European Patent Specification EP 3 495 381 B1, published April 1, 2026. Title: Silk protein coatings. Applicant: AMsilk GmbH. The sequence listing filed with the application follows.

SEQUENCE LISTING (44 sequences)

SEQ ID NO: 1 - protein, 636 aa, Araneus diadematus
  PEPTIDE (1)..(636): ADF-3
ARAGSGQQGPGQQGPGQQGPGQQGPYGPGASAAAAAAGGYGPGSGQQGPSQQGPGQQGPGGQGPYGPGASAAAAAAGGYGPGSGQQGPGGQGPYGPGSSAAAAAAGGNGPGSGQQGAGQQGPGQQGPGASAAAAAAGGYGPGSGQQGPGQQGPGGQGPYGPGASAAAAAAGGYGPGSGQGPGQQGPGGQGPYGPGASAAAAAAGGYGPGSGQQGPGQQGPGQQGPGGQGPYGPGASAAAAAAGGYGPGYGQQGPGQQGPGGQGPYGPGASAASAASGGYGPGSGQQGPGQQGPGGQGPYGPGASAAAAAAGGYGPGSGQQGPGQQGPGQQGPGQQGPGGQGPYGPGASAAAAAAGGYGPGSGQQGPGQQGPGQQGPGQQGPGQQGPGQQGPGQQGPGQQGPGQQGPGGQGAYGPGASAAAGAAGGYGPGSGQQGPGQQGPGQQGPGQQGPGQQGPGQQGPGQQGPGQQGPYGPGASAAAAAAGGYGPGSGQQGPGQQGPGQQGPGGQGPYGPGAASAAVSVGGYGPQSSSVPVASAVASRLSSPAASSRVSSAVSSLVSSGPTKHAALSNTISSVVSQVSASNPGLSGCDVLVQALLEVVSALVSILGSSSIGQINYGASAQYTQMVGQSVAQALA

SEQ ID NO: 2 - protein, 410 aa, Araneus diadematus
  PEPTIDE (1)..(410): ADF-4
AGSSAAAAAAASGSGGYGPENQGPSGPVAYGPGGPVSSAAAAAAAGSGPGGYGPENQGPSGPGGYGPGGSGSSAAAAAAAASGPGGYGPGSQGPSGPGGSGGYGPGSQGASGPGGPGASAAAAAAAAAASGPGGYGPGSQGPSGPGAYGPGGPGSSAAAAAAAASGPGGYGPGSQGPSGPGVYGPGGPGSSAAAAAAAGSGPGGYGPENQGPSGPGGYGPGGSGSSAAAAAAAASGPGGYGPGSQGPSGPGGSGGYGPGSQGGSGPGASAAAAAAAASGPGGYGPGSQGPSGPGYQGPSGPGAYGPSPSASASVAASVYLRLQPRLEVSSAVSSLVSSGPTNGAAVSGALNSLVSQISASNPGLSGCDALVQALLELVSALVAILSSASIGQVNVSSVSQSTQMISQALS

SEQ ID NO: 3 - protein, 5 aa, Artificial Sequence
  synthetic
  REPEAT (1)..(5): consensus peptide motif
GPGXX

SEQ ID NO: 4 - protein, 5 aa, Araneus diadematus
  VARIANT (4)..(4): Q at position 4 may also be alanine, serine, glycine, tyrosine, proline, or glutamine
  VARIANT (5)..(5): Q at position 5 may also be alanine, serine, glycine, tyrosine, proline, or glutamine
GPGQQ

SEQ ID NO: 5 - protein, 5 aa, Araneus diadematus
  REPEAT (1)..(5): peptide motif (ADF-3)
GPGAS

SEQ ID NO: 6 - protein, 5 aa, Araneus diadematus
  REPEAT (1)..(5): peptide motif (ADF-3)
GPGSG

SEQ ID NO: 7 - protein, 5 aa, Araneus diadematus
  REPEAT (1)..(5): peptide motif (ADF-4)
GPGGY

SEQ ID NO: 8 - protein, 5 aa, Araneus diadematus
  REPEAT (1)..(5): peptide motif (ADF-4)
GPGGP

SEQ ID NO: 9 - protein, 5 aa, Nephila clavipes
  REPEAT (1)..(5): peptide motif (flagelliform protein)
GPGGA

SEQ ID NO: 10 - protein, 5 aa, Arthropoda
  REPEAT (1)..(5): peptide motif (resilin)
GPGGG

SEQ ID NO: 11 - protein, 5 aa, Nephila clavipes
  REPEAT (1)..(5): peptide motif (flagelliform protein)
GPGGS

SEQ ID NO: 12 - protein, 5 aa, Artificial Sequence
  synthetic
  REPEAT (1)..(5): Ax peptide motif
AAAAA

SEQ ID NO: 13 - protein, 6 aa, Araneus diadematus
  REPEAT (1)..(6): Ax peptide motif (ADF 3)
AAAAAA

SEQ ID NO: 14 - protein, 7 aa, Araneus diadematus
  REPEAT (1)..(7): Ax peptide motif (ADF-4)
AAAAAAA

SEQ ID NO: 15 - protein, 8 aa, Araneus diadematus
  REPEAT (1)..(8): Ax peptide motif (ADF-4)
AAAAAAAA

SEQ ID NO: 16 - protein, 9 aa, Artificial Sequence
  synthetic
  REPEAT (1)..(9): Ax peptide motif
AAAAAAAAA

SEQ ID NO: 17 - protein, 10 aa, Araneus diadematus
  REPEAT (1)..(10): Ax peptide motif (ADF-4)
AAAAAAAAAA

SEQ ID NO: 18 - protein, 9 aa, Arthropoda
  REPEAT (1)..(9): peptide motif (based on resilin)
GGRPSDTYG

SEQ ID NO: 19 - protein, 9 aa, Arthropoda
  REPEAT (1)..(9): peptide motif (based on resilin)
GGRPSSSYG

SEQ ID NO: 20 - protein, 24 aa, Artificial Sequence
  synthetic
  DOMAIN (1)..(24): Module A (ADF-3)
GPYGPGASAAAAAAGGYGPGSGQQ

SEQ ID NO: 21 - protein, 35 aa, Artificial Sequence
  synthetic
  DOMAIN (1)..(35): Module C (ADF-4)
GSSAAAAAAAASGPGGYGPENQGPSGPGGYGPGGP

SEQ ID NO: 22 - protein, 20 aa, Artificial Sequence
  synthetic
  DOMAIN (1)..(20): Module Q (ADF-3)
GPGQQGPGQQGPGQQGPGQQ

SEQ ID NO: 23 - protein, 27 aa, Artificial Sequence
  synthetic
  DOMAIN (1)..(27): Module K (flagelliform protein)
GPGGAGGPYGPGGAGGPYGPGGAGGPY

SEQ ID NO: 24 - protein, 28 aa, Artificial Sequence
  synthetic
  DOMAIN (1)..(28): Module sp (flagelliform protein)
GGTTIIEDLDITIDGADGPITISEELTI

SEQ ID NO: 25 - protein, 34 aa, Artificial Sequence
  synthetic
  DOMAIN (1)..(34): Module S (Resilin)
PGSSAAAAAAAASGPGQGQGQGQGQGGRPSDTYG

SEQ ID NO: 26 - protein, 39 aa, Artificial Sequence
  synthetic
  DOMAIN (1)..(39): Module R (Resilin)
SAAAAAAAAGPGGGNGGRPSDTYGAPGGGNGGRPSSSYG

SEQ ID NO: 27 - protein, 18 aa, Artificial Sequence
  synthetic
  DOMAIN (1)..(18): Module X (flagelliform protein)
GGAGGAGGAGGSGGAGGS

SEQ ID NO: 28 - protein, 30 aa, Artificial Sequence
  synthetic
  DOMAIN (1)..(30): Module Y (flagelliform protein)
GPGGAGPGGYGPGGSGPGGYGPGGSGPGGY

SEQ ID NO: 29 - protein, 24 aa, Artificial Sequence
  synthetic
  DOMAIN (1)..(24): Module Ac
GPYGPGASAAAAAAGGYGPGCGQQ

SEQ ID NO: 30 - protein, 24 aa, Artificial Sequence
  synthetic
  DOMAIN (1)..(24): Module Ak
GPYGPGASAAAAAAGGYGPGKGQQ

SEQ ID NO: 31 - protein, 35 aa, Artificial Sequence
  synthetic
  DOMAIN (1)..(35): Module Cc
GSSAAAAAAAASGPGGYGPENQGPCGPGGYGPGGP

SEQ ID NO: 32 - protein, 35 aa, Artificial Sequence
  synthetic
  DOMAIN (1)..(35): Module Ck1
GSSAAAAAAAASGPGGYGPENQGPKGPGGYGPGGP

SEQ ID NO: 33 - protein, 35 aa, Artificial Sequence
  synthetic
  DOMAIN (1)..(35): Module Ck2
GSSAAAAAAAASGPGGYGPKNQGPSGPGGYGPGGP

SEQ ID NO: 34 - protein, 35 aa, Artificial Sequence
  synthetic
  DOMAIN (1)..(35): Module Ckc
GSSAAAAAAAASGPGGYGPKNQGPCGPGGYGPGGP

SEQ ID NO: 35 - protein, 13 aa, Artificial Sequence
  synthetic
  DOMAIN (1)..(13): TAG cys1
GCGGGGGGSGGGG

SEQ ID NO: 36 - protein, 8 aa, Artificial Sequence
  synthetic
  DOMAIN (1)..(8): TAG cys2
GCGGGGGG

SEQ ID NO: 37 - protein, 14 aa, Artificial Sequence
  synthetic
  DOMAIN (1)..(14): TAG cys3
GCGGSGGGGSGGGG

SEQ ID NO: 38 - protein, 13 aa, Artificial Sequence
  synthetic
  DOMAIN (1)..(13): TAG lys1
GKGGGGGGSGGGG

SEQ ID NO: 39 - protein, 8 aa, Artificial Sequence
  synthetic
  DOMAIN (1)..(8): TAG lys2
GKGGGGGG

SEQ ID NO: 40 - protein, 5 aa, Arthropoda
  REPEAT (1)..(5): peptide motif (resilin)
GPGQG

SEQ ID NO: 41 - protein, 124 aa, Artificial Sequence
  based on ADF-3
  DOMAIN (1)..(124): NR3 (ADF-3)
GAASAAVSVGGYGPQSSSAPVASAAASRLSSPAASSRVSSAVSSLVSSGPTNQAALSNTISSVVSQVSASNPGLSGCDVLVQALLEVVSALVSILGSSSIGQINYGASAQYTQMVGQSVAQALA

SEQ ID NO: 42 - protein, 109 aa, Artificial Sequence
  based on ADF-4
  DOMAIN (1)..(109): NR4 (ADF-4)
GAYGPSPSASASVAASRLSSPAASSRVSSAVSSLVSSGPTNGAAVSGALNSLVSQISASNPGLSGCDALVQALLELVSALVAILSSASIGQVNVSSVSQSTQMISQALS

SEQ ID NO: 43 - protein, 747 aa, Araneus diadematus
  PEPTIDE (1)..(747): MaSp I
QGAGAAAAAAGGAGQGGYGGLGGQGAGQGGYGGLGGQGAGQGAGAAAAAAAGGAGQGGYGGLGSQGAGRGGQGAGAAAAAAGGAGQGGYGGLGSQGAGRGGLGGQGAGAAAAAAAGGAGQGGYGGLGNQGAGRGGQGAAAAAAGGAGQGGYGGLGSQGAGRGGLGGQGAGAAAAAAGGAGQGGYGGLGGQGAGQGGYGGLGSQGAGRGGLGGQGAGAAAAAAAGGAGQGGLGGQGAGQGAGASAAAAGGAGQGGYGGLGSQGAGRGGEGAGAAAAAAGGAGQGGYGGLGGQGAGQGGYGGLGSQGAGRGGLGGQGAGAAAAGGAGQGGLGGQGAGQGAGAAAAAAGGAGQGGYGGLGSQGAGRGGLGGQGAGAVAAAAAGGAGQGGYGGLGSQGAGRGGQGAGAAAAAAGGAGQRGYGGLGNQGAGRGGLGGQGAGAAAAAAAGGAGQGGYGGLGNQGAGRGGQGAAAAAGGAGQGGYGGLGSQGAGRGGQGAGAAAAAAVGAGQEGIRGQGAGQGGYGGLGSQGSGRGGLGGQGAGAAAAAAGGAGQGGLGGQGAGQGAGAAAAAAGGVRQGGYGGLGSQGAGRGGQGAGAAAAAAGGAGQGGYGGLGGQGVGRGGLGGQGAGAAAAGGAGQGGYGGVGSGASAASAAASRLSSPQASSRVSSAVSNLVASGPTNSAALSSTISNVVSQIGASNPGLSGCDVLIQALLEVVSALIQILGSSSIGQVNYGSAGQATQIVGQSVYQAL

SEQ ID NO: 44 - protein, 627 aa, Araneus diadematus
  PEPTIDE (1)..(627): MaSp II
PGGYGPGQQGPGGYGPGQQGPSGPGSAAAAAAAAAAGPGGYGPGQQGPGGYGPGQQGPGRYGPGQQGPSGPGSAAAAAAGSGQQGPGGYGPRQQGPGGYGQGQQGPSGPGSAAAASAAASAESGQQGPGGYGPGQQGPGGYGPGQQGPGGYGPGQQGPSGPGSAAAAAAAASGPGQQGPGGYGPGQQGPGGYGPGQQGPSGPGSAAAAAAAASGPGQQGPGGYGPGQQGPGGYGPGQQGLSGPGSAAAAAAAGPGQQGPGGYGPGQQGPSGPGSAAAAAAAAAGPGGYGPGQQGPGGYGPGQQGPSGAGSAAAAAAAGPGQQGLGGYGPGQQGPGGYGPGQQGPGGYGPGSASAAAAAAGPGQQGPGGYGPGQQGPSGPGSASAAAAAAAAGPGGYGPGQQGPGGYAPGQQGPSGPGSASAAAAAAAAGPGGYGPGQQGPGGYAPGQQGPSGPGSAAAAAAAAAGPGGYGPAQQGPSGPGIAASAASAGPGGYGPAQQGPAGYGPGSAVAASAGAGSAGYGPGSQASAAASRLASPDSGARVASAVSNLVSSGPTSSAALSSVISNAVSQIGASNPGLSGCDVLIQALLEIVSACVTILSSSSIGQVNYGAASQFAQVVGQSVLSAF